European Patent Specification EP 4 059 952 B1, published January 8, 2025. Title: Novel primosome assembly protein variant and a method for producing L-lysine using the same. Applicant: CJ CheilJedang Corporation. The sequence listing filed with the application follows.

SEQUENCE LISTING (11 sequences)

SEQ ID NO: 1 - protein, 688 aa, Artificial Sequence
  (R304Q)_primosome assembly protein
MAKTRVPAPEKSVARVLPLLGLPHLDRLFDYRISEDQHDDVQPGVRVRVRFGGRLVDAIVMSRTAQTSHEGKLMWLDRVISPIVVYPPQTAKLIEQLSDRYGGVRSDLIRSALPARHAGAEEADTSTSWESLGEVKEPDLSSWSAYQHGQSFVDAVLAGTTARASWQIAPGDDWALALASLAVKVVKDGGGALLVVPDQRDLDRLEAALRGLVAAKQITVLNSGLGPQARYRRFLSVLSGQGRLIIGTRSAAFAPVKDLKLAVILNDGDDNLVDPRAPYAHAREVLTTRSSLEASSLIIAGHAQTAETQLLVESGWMHNLIAPRDTIRTRMPRIQAVGDSDFQMERDPMARSARLPGIAFHAVRSALERDQPALIQVPRKGYVPTLACGNCRTPARCRHCNGPVGLPQGSSDLAGVPTCRWCGRPDSRFKCQNCGSPKLRAVVLGTERTAEELGRAFPSVRVITSGGNKVVDSVENRASIVVSTPGAEPFVANSPERPEKSEKPEHKGAYGALLLLDTWALMGRQDLRAMEDALHKWAAAATLVHSHLHQGQVIVVADPSFPAVQSLIRWDMAGAAAQELASRREVMFPPSVHMAAIDGATAALESFLDLAELPDHAEVLGPVDLPPGVSLPGEYDEQRFGPPQRLLIRTPLGPRSELGRALRSAQVARAVRKNDLPLRIQMDPIHIG

SEQ ID NO: 2 - DNA, 2067 bp, Artificial Sequence
  (R304Q)_NCgl1540
atggcaaaaacccgcgtccccgctcctgaaaagtcggtggcgcgggttttacctcttttggggttacctcacctggatcgactgtttgattaccgcatcagcgaagaccaacacgatgatgtgcaacctggcgtgcgggtgcgcgtgcgttttggtggacgtttagttgatgccatcgtgatgtcacgcaccgcgcaaacctcgcacgagggaaagctgatgtggctggatcgggtgatttcgccgatcgtggtgtatccacctcaaacagcaaagctaattgagcaactcagtgatcgctatggcggggtacgttcggatctcatccgttcggcgctaccggcgcggcatgctggggcagaagaggcagatacctccacgtcgtgggagtcattgggtgaggttaaagaacccgatttatcgtcgtggtctgcgtatcagcatggtcaatcatttgttgacgccgtcttggcgggaacaactgcgcgggcgtcatggcagattgctcccggagatgattgggcgctggctttggcttctttggcggtcaaggttgtcaaagacggcggcggagcgcttctcgtagtgcctgatcagcgcgatctcgaccgcttggaagctgcgcttcgaggtttggttgcggcgaaacaaatcactgtgcttaattcaggtcttggtccgcaggcacgatatcggcgtttcctatcggtactcagtgggcagggacgactgattattggaaccagaagtgccgcttttgcacccgtgaaggatctgaaactggccgtcattttaaatgatggcgacgacaacctcgttgatcctagagcgccctatgcccacgccagggaagtgctgaccacgcgttccagtttggaagcaagctccttgattattgcgggacatgcgcagaccgcggaaacccaattgctggtggaatcgggatggatgcacaatctcatcgcaccgagggataccattcgcactaggatgccgcgtattcaggcagtgggcgattccgatttccagatggaacgcgatccaatggcccgatcagcgcggctgcctggcattgcgtttcatgcggtgcgcagcgccttagaacgtgatcaaccagcgcttatccaggtaccaaggaaaggctacgtgccaaccttggcgtgtggaaactgccgcaccccagcgcggtgccggcactgtaatgggcctgtgggacttccccagggaagctctgatctagcgggagtgcccacttgccgatggtgcggacgccctgattcgcggtttaagtgccaaaactgcggctctccaaaactgcgtgctgtggtgctgggaacggaacgcacagcagaagaactgggccgcgcgttcccgtctgtgcgggtaattacctctggtggcaacaaggtggtggattcggtggaaaaccgagccagcattgtggtgtccacgccaggtgcagaaccttttgtggccaactcgccggagagaccagagaaatcggagaaaccagagcacaagggcgcttacggtgccttgttattgctggatacctgggcgttgatgggtcggcaagatctgcgcgccatggaggacgcgctgcacaagtgggcagcggcggccacgctggtgcattctcatctgcaccagggtcaagtcatcgtggttgcagatccatcgtttcctgctgtgcaatcgttgattcggtgggatatggcaggtgctgcagcgcaagagttggctagccgacgcgaggttatgttcccgccttctgtacacatggcagcaatcgatggggctaccgctgcattggaaagtttcttggatttggcggagcttcccgatcatgctgaagtcctcggccctgttgatctgccaccgggtgtgagtttgcctggtgaatatgatgagcagcgctttggtccgccgcagcgccttctcatcagaactccattgggaccgcggtctgagttgggtagagcgctgcgctcagcccaggtggcgcgtgcggtgaggaagaatgatttgccgttgcgtattcagatggatccgattcacatcggataa

SEQ ID NO: 3 - protein, 688 aa, Artificial Sequence
  (WT)_primosome assembly protein
MAKTRVPAPEKSVARVLPLLGLPHLDRLFDYRISEDQHDDVQPGVRVRVRFGGRLVDAIVMSRTAQTSHEGKLMWLDRVISPIVVYPPQTAKLIEQLSDRYGGVRSDLIRSALPARHAGAEEADTSTSWESLGEVKEPDLSSWSAYQHGQSFVDAVLAGTTARASWQIAPGDDWALALASLAVKVVKDGGGALLVVPDQRDLDRLEAALRGLVAAKQITVLNSGLGPQARYRRFLSVLSGQGRLIIGTRSAAFAPVKDLKLAVILNDGDDNLVDPRAPYAHAREVLTTRSSLEASSLIIAGHARTAETQLLVESGWMHNLIAPRDTIRTRMPRIQAVGDSDFQMERDPMARSARLPGIAFHAVRSALERDQPALIQVPRKGYVPTLACGNCRTPARCRHCNGPVGLPQGSSDLAGVPTCRWCGRPDSRFKCQNCGSPKLRAVVLGTERTAEELGRAFPSVRVITSGGNKVVDSVENRASIVVSTPGAEPFVANSPERPEKSEKPEHKGAYGALLLLDTWALMGRQDLRAMEDALHKWAAAATLVHSHLHQGQVIVVADPSFPAVQSLIRWDMAGAAAQELASRREVMFPPSVHMAAIDGATAALESFLDLAELPDHAEVLGPVDLPPGVSLPGEYDEQRFGPPQRLLIRTPLGPRSELGRALRSAQVARAVRKNDLPLRIQMDPIHIG

SEQ ID NO: 4 - DNA, 2067 bp, Artificial Sequence
  (WT)_NCgl1540
atggcaaaaacccgcgtccccgctcctgaaaagtcggtggcgcgggttttacctcttttggggttacctcacctggatcgactgtttgattaccgcatcagcgaagaccaacacgatgatgtgcaacctggcgtgcgggtgcgcgtgcgttttggtggacgtttagttgatgccatcgtgatgtcacgcaccgcgcaaacctcgcacgagggaaagctgatgtggctggatcgggtgatttcgccgatcgtggtgtatccacctcaaacagcaaagctaattgagcaactcagtgatcgctatggcggggtacgttcggatctcatccgttcggcgctaccggcgcggcatgctggggcagaagaggcagatacctccacgtcgtgggagtcattgggtgaggttaaagaacccgatttatcgtcgtggtctgcgtatcagcatggtcaatcatttgttgacgccgtcttggcgggaacaactgcgcgggcgtcatggcagattgctcccggagatgattgggcgctggctttggcttctttggcggtcaaggttgtcaaagacggcggcggagcgcttctcgtagtgcctgatcagcgcgatctcgaccgcttggaagctgcgcttcgaggtttggttgcggcgaaacaaatcactgtgcttaattcaggtcttggtccgcaggcacgatatcggcgtttcctatcggtactcagtgggcagggacgactgattattggaaccagaagtgccgcttttgcacccgtgaaggatctgaaactggccgtcattttaaatgatggcgacgacaacctcgttgatcctagagcgccctatgcccacgccagggaagtgctgaccacgcgttccagtttggaagcaagctccttgattattgcgggacatgcgcggaccgcggaaacccaattgctggtggaatcgggatggatgcacaatctcatcgcaccgagggataccattcgcactaggatgccgcgtattcaggcagtgggcgattccgatttccagatggaacgcgatccaatggcccgatcagcgcggctgcctggcattgcgtttcatgcggtgcgcagcgccttagaacgtgatcaaccagcgcttatccaggtaccaaggaaaggctacgtgccaaccttggcgtgtggaaactgccgcaccccagcgcggtgccggcactgtaatgggcctgtgggacttccccagggaagctctgatctagcgggagtgcccacttgccgatggtgcggacgccctgattcgcggtttaagtgccaaaactgcggctctccaaaactgcgtgctgtggtgctgggaacggaacgcacagcagaagaactgggccgcgcgttcccgtctgtgcgggtaattacctctggtggcaacaaggtggtggattcggtggaaaaccgagccagcattgtggtgtccacgccaggtgcagaaccttttgtggccaactcgccggagagaccagagaaatcggagaaaccagagcacaagggcgcttacggtgccttgttattgctggatacctgggcgttgatgggtcggcaagatctgcgcgccatggaggacgcgctgcacaagtgggcagcggcggccacgctggtgcattctcatctgcaccagggtcaagtcatcgtggttgcagatccatcgtttcctgctgtgcaatcgttgattcggtgggatatggcaggtgctgcagcgcaagagttggctagccgacgcgaggttatgttcccgccttctgtacacatggcagcaatcgatggggctaccgctgcattggaaagtttcttggatttggcggagcttcccgatcatgctgaagtcctcggccctgttgatctgccaccgggtgtgagtttgcctggtgaatatgatgagcagcgctttggtccgccgcagcgccttctcatcagaactccattgggaccgcggtctgagttgggtagagcgctgcgctcagcccaggtggcgcgtgcggtgaggaagaatgatttgccgttgcgtattcagatggatccgattcacatcggataa

SEQ ID NO: 5 - DNA, 35 bp, Artificial Sequence
  NCgl1540_1F
tcgagctcggtacccacccgatttatcgtcgtggt

SEQ ID NO: 6 - DNA, 41 bp, Artificial Sequence
  NCgl1540_2R
gcaattgggtttccgcggtctgcgcatgtcccgcaataatc

SEQ ID NO: 7 - DNA, 41 bp, Artificial Sequence
  NCgl1540_3F
gattattgcgggacatgcgcagaccgcggaaacccaattgc

SEQ ID NO: 8 - DNA, 35 bp, Artificial Sequence
  NCgl1540_4R
ctctagaggatccccccaccttgttgccaccagag

SEQ ID NO: 9 - DNA, 20 bp, Artificial Sequence
  NCgl1540_5F
acccgatttatcgtcgtggt

SEQ ID NO: 10 - DNA, 20 bp, Artificial Sequence
  NCgl1540_6R
ccaccttgttgccaccagag

SEQ ID NO: 11 - DNA, 5803 bp, Artificial Sequence
  pDCM2_plasmid
gttcgcttgctgtccataaaaccgcccagtctagctatcgccatgtaagcccactgcaagctacctgctttctctttgcgcttgcgttttcccttgtccagatagcccagtagctgacattcatccggggtcagcaccgtttctgcggactggctttctacgtgttccgcttcctttagcagcccttgcgccctgagtgcttgcggcagcgtgaagctagcttttatcgccattcgccattcaggctgcgcaactgttgggaagggcgatcggtgcgggcctcttcgctattacgccagctggcgaaagggggatgtgctgcaaggcgattaagttgggtaacgccagggttttcccagtcacgacgttgtaaaacgacggccagtgaattcgagctcggtacccggggatcctctagagtcgacctgcaggcatgcaagcttggcgtaatcatggtcatagctgtttcctgtgtgaaattgttatccgctcacaattccacacaacatacgagccggaagcataaagtgtaaagcctggggtgcctaatgagtgagctaactcacattaattgcgttgcgctcactgcccgctttccagtcgggaaacctgtcgtgccagctgcattaatgaatcggccaacgcgcggggagaggcggtttgcgtattgggcgctcttccgcttcctcgctcactgactcgctgcgctcggtcgttcggctgcggcgagcggtatcagctcactcaaaggcggtaatacggttatccacagaatcaggggataacgcaggaaagaacatgtgagcaaaaggccagcaaaaggccaggaaccgtaaaaaggccgcgttgctggcgtttttccataggctccgcccccctgacgagcatcacaaaaatcgacgctcaagtcagaggtggcgaaacccgacaggactataaagataccaggcgtttccccctggaagctccctcgtgcgctctcctgttccgaccctgccgcttaccggatacctgtccgcctttctcccttcgggaagcgtggcgctttctcaatgctcacgctgtaggtatctcagttcggtgtaggtcgttcgctccaagctgggctgtgtgcacgaaccccccgttcagcccgaccgctgcgccttatccggtaactatcgtcttgagtccaacccggtaagacacgacttatcgccactggcagcagccactggtaacaggattagcagagcgaggtatgtaggcggtgctacagagttcttgaagtggtggcctaactacggctacactagaaggacagtatttggtatctgcgctctgctgaagccagttaccttcggaaaaagagttggtagctcttgatccggcaaacaaaccaccgctggtagcggtggtttttttgtttgcaagcagcagattacgcgcagaaaaaaaggatctcaagaagatcctttgatcttttctacggggtctgacgctcagtggaacgaaaactcacgttaagggattttggtcatgagattatcaaaaaggatcttcacctagatccttttggggtgggcgaagaactccagcatgagatccccgcgctggaggatcatccagccctgatagaaacagaagccactggagcacctcaaaaacaccatcatacactaaatcagtaagttggcagcatcacccgacgcactttgcgccgaataaatacctgtgacggaagatcacttcgcagaataaataaatcctggtgtccctgttgataccgggaagccctgggccaacttttggcgaaaatgagacgttgatcggcacgtaagaggttccaactttcaccataatgaaataagatcactaccgggcgtattttttgagttatcgagattttcaggagctgatagaaacagaagccactggagcacctcaaaaacaccatcatacactaaatcagtaagttggcagcatcacccgacgcactttgcgccgaataaatacctgtgacggaagatcacttcgcagaataaataaatcctggtgtccctgttgataccgggaagccctgggccaacttttggcgaaaatgagacgttgatcggcacgtaagaggttccaactttcaccataatgaaataagatcactaccgggcgtattttttgagttatcgagattttcaggagctctttggcatcgtctctcgcctgtcccctcagttcagtaatttcctgcatttgcctgtttccagtcggtagatattccacaaaacagcagggaagcagcgcttttccgctgcataaccctgcttcggggtcattatagcgattttttcggtatatccatcctttttcgcacgatatacaggattttgccaaagggttcgtgtagactttccttggtgtatccaacggcgtcagccgggcaggataggtgaagtaggcccacccgcgagcgggtgttccttcttcactgtcccttattcgcacctggcggtgctcaacgggaatcctgctctgcgaggctggccggctaccgccggcgtaacagatgagggcaagcggatggctgatgaaaccaagccaaccaggaagggcagcccacctatcaaggtgtactgccttccagacgaacgaagagcgattgaggaaaaggcggcggcggccggcatgagcctgtcggcctacctgctggccgtcggccagggctacaaaatcacgggcgtcgtggactatgagcacgtccgcgagggcgtcccggaaaacgattccgaagcccaacctttcatagaaggcggcggtggaatcgaaatctcgtgatggcaggttgggcgtcgcttggtcggtcatttcgaaaaaggttaggaatacggttagccatttgcctgcttttatatagttcantatgggattcacctttatgttgataagaaataaaagaaaatgccaataggatatcggcattttcttttgcgtttttatttgttaactgttaattgtccttgttcaaggatgctgtctttgacaacagatgttttcttgcctttgatgttcagcaggaagctcggcgcaaacgttgattgtttgtctgcgtagaatcctctgtttgtcatatagcttgtaatcacgacattgtttcctttcgcttgaggtacagcgaagtgtgagtaagtaaaggttacatcgttaggcggatcaagatccatttttaacacaaggccagttttgttcagcggcttgtatgggccagttaaagaattagaaacataaccaagcatgtaaatatcgttagacgtaatgccgtcaatcgtcatttttgatccgcgggagtcagtgaacaggtaccatttgccgttcattttaaagacgttcgcgcgttcaatttcatctgttactgtgttagatgcaatcagcggtttcatcacttttttcagtgtgtaatcatcgtttagctcaatcataccgagagcgccgtttgctaactcagccgtgcgttttttatcgctttgcagaagtttttgactttcttgacggaagaatgatgtgcttttgccatagtatgctttgttaaataaagattcttcgccttggtagccatcttcagttccagtgtttgcttcaaatactaagtatttgtggcctttatcttctacgtagtgaggatctctcagcgtatggttgtcgcctgagctgtagttgccttcatcgatgaactgctgtacattttgatacgtttttccgtcaccgtcaaagattgatttataatcctctacaccgttgatgttcaaagagctgtctgatgctgatacgttaacttgtgcagttgtcagtgtttgtttgccgtaatgtttaccggagaaatcagtgtagaataaacggatttttccgtcagatgtaaatgtggctgaacctgaccattcttgtgtttggtcttttaggatagaatcatttgcatcgaatttgtcgctgtctttaaagacgcggccagcgtttttccagctgtcaatagaagtttcgccgactttttgatagaacatgtaaatcgatgtgtcatccgcatttttaggatctccggctaatgcaaagacgatgtggtagccgtgatagtttgcgacagtgccgtcagcgttttgtaatggccagctgtcccaaacgtccaggccttttgcagaagagatatttttaattgtggacgaatcaaattcagaaacttgatatttttcatttttttgctgttcagggatttgcagcatatcatggcgtgtaatatgggaaatgccgtatgtttccttatatggcttttggttcgtttctttcgcaaacgcttgagttgcgcctcctgccagcagtgcggtagtaaaggttaatactgttgcttgttttgcaaactttttgatgttcatcgttcatgtctccttttttatgtactgtgttagcggtctgcttcttccagccctcctgtttgaagatggcaagttagttacgcacaataaaaaaagacctaaaatatgtaaggggtgacgccaaagtatacactttgccctttacacattttaggtcttgcctgctttatcagtaacaaacccgcgcgatttacttttcgacctcattctattagactctcgtttggattgcaactggtctattttcctcttttgtttgatagaaaatcataaaaggatttgcagactacgggcctaaagaactaaaaaatctatctgtttcttttcattctctgtattttttatagtttctgttgcatgggcataaagttgcctttttaatcacaattcagaaaatatcataatatctcatttcactaaataatagtgaacggcaggtatatgtgatgggttaaaaaggatcaccccagagtcccgctcagaagaactcgtcaagaaggcgatagaaggcgatgcgctgcgaatcgggagcggcgataccgtaaagcacgaggaagcggtcagcccattcgccgccaagctcttcagcaatatcacgggtagccaacgctatgtcctgatagcggtccgccacacccagccggccacagtcgatgaatccagaaaagcggccattttccaccatgatattcggcaagcaggcatcgccatgggtcacgacgagatcctcgccgtcgggcatccgcgccttgagcctggcgaacagttcggctggcgcgagcccctgatgctcttcgtccagatcatcctgatcgacaagaccggcttccatccgagtacgtgctcgctcgatgcgatgtttcgcttggtggtcgaatgggcaggtagccggatcaagcgtatgcagccgccgcattgcatcagccatgatggatactttctcggcaggagcaaggtgagatgacaggagatcctgccccggcacttcgcccaatagcagccagtcccttcccgcttcagtgacaacgtcgagacagctgcgcaaggaacgcccgtcgtggccagccacgatagccgcgctgcctcgtcttggagttcattcagggcaccggacaggtcggtcttgacaaaaagaaccgggcgcccctgcgctgacagccggaacacggcggcatcagagcagccgattgtctgttgtgcccagtcatagccgaatagcctctccacccaagcggccggagaacctgcgtgcaatccatcttgttcaatcatgcgaaacgatcctcatcctgtctcttgatcagatcttgatcccctgcgccatcagatccttggcggcaagaaagccatccagtttactttgcagggcttcccaaccttaccagagggcgccccagctggcaattccg